European Patent Specification EP 4 214 308 B1, published November 20, 2024. Title: Generation of a high producing recombinant Chinese hamster ovary cell line for therapeutic protein production. Applicant: SANOFI. The sequence listing filed with the application follows.

SEQUENCE LISTING (36 sequences)

SEQ ID NO: 1 - DNA, 1188 bp, Cricetulus griseus
atggcttggcggcagatgcggaagagagccctggacgccgctatcatcctgggaggcggaggcctgctgttcacctcttacctgacagccaccggcgacgaccacttctacgccgagtacctgatgcctgccctgcagagactgctggaccctgagtctgcccaccggctggccatcagattcacctccctgggcctgctgcccagagccaccttccaggactccgacatgctggaagtgcgggtgctgggccacaagttcagaaaccccgtgggaatcgccgctggcttcgacaagcacggcgaggctgtggacggcctgtacaagctgggcttcggcttcgtggaagtgggctccgtgacaccccagccccaggaaggcaaccccagacctagagtgttccggctgcctgaggaccaggccgtgatcaacagatacggcttcaactcccacggcctgtccgtggtggaacaccggctgagagccagacagcagaagcagaacaagctgaccgccgacggcctgcccctgggcatcaatctgggcaagaacaagacctccgaggacgctgccgccgactacgtggaaggcgtgcgagtgctgggacctctggccgattacctggtcgtgaacgtgtcctcccccaacaccgctggcctgagaagcctgcagggaaaggccgagctgagaaggctgctggccaaggtgctgcaggaacgggacgctctgaagggcgcccagaaacctgccgtgctcgtgaagatcgcccctgacctgaccgcccaggacaaagaggatatcgcctccgtggccagagagctgggcatcgacggactgatcgtgaccaacaccaccgtgtctcggcctaccggactgcagggcgctctgagatctgagatgggcggcctgtctggcaagcctctgagggacctgtccacccagaccatcagagagatgtacaccctgacccagggccggatccccatcattggagtgggcggagtgtcctctggccaggacgccctggaaaagatccaggctggcgcctctctggtgcagctgtataccgccctgacctttctgggccctcccgtggtggtgcgagtgaagagagaactggaagccctgctgaaagagcggggcttcaacaccgtgaccgaggccatcggcgctgaccacagaagatga

SEQ ID NO: 2 - protein, 395 aa, Cricetulus griseus
MAWRQMRKRALDAAIILGGGGLLFTSYLTATGDDHFYAEYLMPALQRLLDPESAHRLAIRFTSLGLLPRATFQDSDMLEVRVLGHKFRNPVGIAAGFDKHGEAVDGLYKLGFGFVEVGSVTPQPQEGNPRPRVFRLPEDQAVINRYGFNSHGLSVVEHRLRARQQKQNKLTADGLPLGINLGKNKTSEDAAADYVEGVRVLGPLADYLVVNVSSPNTAGLRSLQGKAELRRLLAKVLQERDALKGAQKPAVLVKIAPDLTAQDKEDIASVARELGIDGLIVTNTTVSRPTGLQGALRSEMGGLSGKPLRDLSTQTIREMYTLTQGRIPIIGVGGVSSGQDALEKIQAGASLVQLYTALTFLGPPVVVRVKRELEALLKERGFNTVTEAIGADHRR

SEQ ID NO: 3 - DNA, 1188 bp, Homo sapiens
atggcttggcggcacctgaagaagagggcccaggacgccgtgatcatcctgggaggcggaggcctgctgttcgcctcttacctgatggctaccggcgacgagcggttctacgccgagcatctgatgcccacactgcagggcctgctggaccctgagtctgcccatagactggccgtgcggttcacctccctgggactgctgcctagagcccggttccaggactccgacatgctggaagtgcgggtgctgggccacaagttcagaaaccccgtgggaatcgccgctggcttcgacaagcacggcgaggctgtggacggcctgtacaagatgggcttcggcttcgtggaaatcggctccgtgacccccaagccccaggaaggcaaccccagacctcgggtgttcagactgcctgaggaccaggctgtgatcaacagatacggcttcaactcccacggcctgtccgtggtggaacaccggctgagagccagacagcagaagcaggccaagctgaccgaggatggcctgcctctgggagtgaacctgggcaagaacaagacctccgtggacgccgccgaggattacgctgaaggcgtgcgagtgctgggacccctggctgattacctggtcgtgaacgtgtcctcccccaacaccgctggcctgagatctctgcagggcaaggccgagctgcggagactgctgacaaaggtgctgcaggaacgcgacggcctgcggagagtgcatagacctgccgtgctcgtgaagatcgcccccgacctgaccagccaggacaaagaggatatcgcctccgtcgtgaaagagctgggcatcgacggactgatcgtgaccaacaccaccgtgtctaggcctgccggactgcagggggctctgagatctgaaaccggcggactgtccggcaagcctctgagggatctgtccacccagaccatcagagagatgtacgccctgacccagggccgggtgccaatcattggagtgggcggagtgtcctccggccaggatgccctggaaaagatcagagccggcgcttccctggtgcagctgtacaccgctctgaccttttggggccctcccgtcgtgggcaaagtgaagagagagctggaagccctgctgaaagagcagggatttggcggcgtgaccgatgccatcggcgctgaccacagaagatga

SEQ ID NO: 4 - protein, 395 aa, Homo sapiens
MAWRHLKKRAQDAVIILGGGGLLFASYLMATGDERFYAEHLMPTLQGLLDPESAHRLAVRFTSLGLLPRARFQDSDMLEVRVLGHKFRNPVGIAAGFDKHGEAVDGLYKMGFGFVEIGSVTPKPQEGNPRPRVFRLPEDQAVINRYGFNSHGLSVVEHRLRARQQKQAKLTEDGLPLGVNLGKNKTSVDAAEDYAEGVRVLGPLADYLVVNVSSPNTAGLRSLQGKAELRRLLTKVLQERDGLRRVHRPAVLVKIAPDLTSQDKEDIASVVKELGIDGLIVTNTTVSRPAGLQGALRSETGGLSGKPLRDLSTQTIREMYALTQGRVPIIGVGGVSSGQDALEKIRAGASLVQLYTALTFWGPPVVGKVKRELEALLKEQGFGGVTDAIGADHRR

SEQ ID NO: 5 - DNA, 1122 bp, Homo sapiens
atgaccacctccgcctccagccacctgaacaagggcatcaaacaggtgtacatgagcctgccccagggcgagaaggtgcaggccatgtacatctggatcgacggcaccggcgagggactgcggtgcaagaccagaaccctggactccgagcctaagtgcgtggaagaactgcccgagtggaacttcgacggctcctccaccctgcagtccgagggctccaactccgacatgtacctggtgcctgccgccatgttccgggaccctttccggaaggaccccaacaagctggtgctgtgcgaggtgttcaagtacaacagacggcctgccgagacaaacctgcggcatacctgcaagcggatcatggacatggtgtccaaccagcacccttggtttggcatggaacaggagtacaccctgatgggcaccgacggccaccccttcggctggccttctaacggcttccctggcccccagggcccctactattgtggcgtgggcgccgaccgggcctacggcagagatatcgtggaagcccactaccgggcctgcctgtacgccggagtgaagatcgccggcaccaacgccgaagtgatgcccgcccagtgggagttccagatcggcccttgcgagggcatctccatgggcgatcacctgtgggtggcccggttcatcctgcacagagtgtgcgaggacttcggcgtgatcgccaccttcgaccccaagcccatccccggcaactggaacggcgctggctgccacaccaacttctccaccaaggccatgcgggaagagaacggcctgaagtacatcgaggaagccatcgagaagctgtccaagcggcaccagtaccacatcagagcctacgaccctaagggcggcctggacaacgccagaaggctgaccggctttcacgagacatccaacatcaacgacttctctgccggcgtggccaacagatccgcctccatccggatccctagaaccgtgggccaggaaaagaagggctacttcgaggacagacggccctccgccaactgcgacccctttagcgtgaccgaggccctgatccggacctgcctgctgaacgagacaggcgacgagcccttccagtacaagaactga

SEQ ID NO: 6 - protein, 373 aa, Homo sapiens
MTTSASSHLNKGIKQVYMSLPQGEKVQAMYIWIDGTGEGLRCKTRTLDSEPKCVEELPEWNFDGSSTLQSEGSNSDMYLVPAAMFRDPFRKDPNKLVLCEVFKYNRRPAETNLRHTCKRIMDMVSNQHPWFGMEQEYTLMGTDGHPFGWPSNGFPGPQGPYYCGVGADRAYGRDIVEAHYRACLYAGVKIAGTNAEVMPAQWEFQIGPCEGISMGDHLWVARFILHRVCEDFGVIATFDPKPIPGNWNGAGCHTNFSTKAMREENGLKYIEEAIEKLSKRHQYHIRAYDPKGGLDNARRLTGFHETSNINDFSAGVANRSASIRIPRTVGQEKKGYFEDRRPSANCDPFSVTEALIRTCLLNETGDEPFQYKN

SEQ ID NO: 7 - DNA, 1122 bp, Canis lupus
atggccacctccgcctccagccacctgaacaagggcatcaaacaggtgtacatgagcctgccccagggcgagaaggtgcaggccatgtacatctggatcgacggcaccggcgagggactgcggtgcaagaccagaaccctggactccgagcccaagggcgtggaagaactgcccgagtggaacttcgacggctcctccaccttccagtccgagggctccaactccgacatgtacctggtgcctgccgccatgttccgggaccctttccggaaggaccccaacaagctggtgttctgcgaggtgttcaagtacaaccggaagcccgccgagacaaacctgcggcatacctgcaagcggatcatggacatggtgtccaaccagcacccttggtttggcatggaacaggagtacaccctgatgggcaccgacggccaccccttcggctggccttctaacggcttccctggcccccagggcccctactattgtggcgtgggcgccgacaaggcctacggcagagacatcgtggaagcccactaccgggcctgcctgtacgccggcatcaagatcgctggcaccaacgccgaagtgatgcccgcccagtgggagttccagatcggcccttgcgagggcatcgacatgggcgatcacctgtgggtggcccggttcatcctgcacagagtgtgcgaggacttcggcgtgatcgccaccttcgaccccaagcccatccccggcaactggaacggcgctggctgccacaccaacttctccaccaaggccatgcgggaagagaacggcctgaagtacatcgaggaatccatcgagaagctgtccaagcggcaccagtaccacatccgggcctacgaccccaagggcggcctggataacgccagacggctgaccggcttccacgagacatccaacatcaacgacttctctgccggcgtggccaacagaggcgcctccatccggatcccccggaccgtgggccaggaaaagaagggctacttcgaggacagacggccctccgccaactgcgacccctttagcgtgaccgaggccctgatccggacctgcctgctgaacgagacaggcgacgagcccttccagtacaagaactga

SEQ ID NO: 8 - protein, 373 aa, Canis lupus
MATSASSHLNKGIKQVYMSLPQGEKVQAMYIWIDGTGEGLRCKTRTLDSEPKGVEELPEWNFDGSSTFQSEGSNSDMYLVPAAMFRDPFRKDPNKLVFCEVFKYNRKPAETNLRHTCKRIMDMVSNQHPWFGMEQEYTLMGTDGHPFGWPSNGFPGPQGPYYCGVGADKAYGRDIVEAHYRACLYAGIKIAGTNAEVMPAQWEFQIGPCEGIDMGDHLWVARFILHRVCEDFGVIATFDPKPIPGNWNGAGCHTNFSTKAMREENGLKYIEESIEKLSKRHQYHIRAYDPKGGLDNARRLTGFHETSNINDFSAGVANRGASIRIPRTVGQEKKGYFEDRRPSANCDPFSVTEALIRTCLLNETGDEPFQYKN

SEQ ID NO: 9 - protein, 373 aa, Cricetulus griseus
MATSASSHLNKGIKQMYMSLPQGEKVQAMYIWVDGTGEGLRCKTRTLDCEPKCVEELPEWNFDGSSTFQSESSNSDMYLSPVAMFRDPFRKEPNKLVFCEVFKYNQKPAETNLRHTCKRIMDMVSNQHPWFGMEQEYTLLGTDGHPFGWPSDGFPGPQGLYYCGVGADKAYRRDIMEAHYRACLYAGVKITGTYAEVKHAQWEFQIGPCEGIRMGDHLWVARFILHRVCKDFGVIATFDSKPIPGNWNGAGCHTNFSTKTMREENGLKHIKEAIEKLSKRHRYHIRAYDPKGGLDNARRLTGFHKTSNINDFSAGVADRSASIRIPRTVGQEKKGYFEARCPSANCDPFAVTEAIVRTCLLNETGDQPFQYKN

SEQ ID NO: 10 - DNA, 20 bp, Artificial Sequence
  corresponding piece of DNA for generating DHODH gRNA
ggatgcagccatcatccttg

SEQ ID NO: 11 - DNA, 25 bp, Artificial Sequence
  oligonucleotide used for obtaining DHODH gRNA (Sequence1')
ggatgcagccatcatccttggtttt

SEQ ID NO: 12 - DNA, 25 bp, Artificial Sequence
  oligonucleotide used for obtaining DHODH gRNA (Sequence1')
caaggatgatggctgcatcccggtg

SEQ ID NO: 13 - DNA, 25 bp, Artificial Sequence
  oligonucleotide used for obtaining  DHODH gRNA (Sequence2')
gatgcagccatcatccttgggtttt

SEQ ID NO: 14 - DNA, 25 bp, Artificial Sequence
  oligonucleotide used for obtaining DHODH gRNA (Sequence2')
ccaaggatgatggctgcatccggtg

SEQ ID NO: 15 - DNA, 25 bp, Artificial Sequence
  oligonucleotide used for obtaining DHODH gRNA (Sequence3')
gcagccatcatccttggggggtttt

SEQ ID NO: 16 - DNA, 25 bp, Artificial Sequence
  oligonucleotide used for obtaining DHODH gRNA (Sequence3')
cccccaaggatgatggctgccggtg

SEQ ID NO: 17 - DNA, 25 bp, Artificial Sequence
  oligonucleotide used for obtaining  DHODH gRNA (Sequence4')
gccatcatccttgggggagggtttt

SEQ ID NO: 18 - DNA, 25 bp, Artificial Sequence
  oligonucleotide used for obtaining DHODH gRNA (Sequence4')
cctcccccaaggatgatggccggtg

SEQ ID NO: 19 - DNA, 25 bp, Artificial Sequence
  oligonucleotide used for obtaining DHODH gRNA (Sequence5')
gctattcgcttcacgtccctgtttt

SEQ ID NO: 20 - DNA, 25 bp, Artificial Sequence
  oligonucleotide used for obtaining DHODH gRNA (Sequence5')
agggacgtgaagcgaatagccggtg

SEQ ID NO: 21 - DNA, 25 bp, Artificial Sequence
  oligonucleotide used for obtaining DHODH gRNA (Sequence6')
gcctctacaaactgggctttgtttt

SEQ ID NO: 22 - DNA, 25 bp, Artificial Sequence
  oligonucleotide used for obtaining DHODH gRNA (Sequence6')
aaagcccagtttgtagaggccggtg

SEQ ID NO: 23 - DNA, 25 bp, Artificial Sequence
  oligonucleotide used for obtaining DHODH gRNA (Sequence7')
ggctttgggtttgtcgaggtgtttt

SEQ ID NO: 24 - DNA, 25 bp, Artificial Sequence
  oligonucleotide used for obtaining DHODH gRNA (Sequence7')
acctcgacaaacccaaagcccggtg

SEQ ID NO: 25 - DNA, 25 bp, Artificial Sequence
  oligonucleotide used for obtaining DHODH gRNA (Sequence8')
gctggtctgaggagcctacagtttt

SEQ ID NO: 26 - DNA, 25 bp, Artificial Sequence
  oligonucleotide used for obtaining DHODH gRNA (Sequence8')
tgtaggctcctcagaccagccggtg

SEQ ID NO: 27 - DNA, 14437 bp, Cricetulus griseus
  misc_feature (1992)..(2015): target of plasmids pBH6840 KO DHODH SEQ1 and pBH6841 KO DHODH SEQ4
  misc_feature (2129)..(2147): target of plasmids pBH6842 KO DHODH SEQ5
  misc_feature (4015)..(4047): target of plasmids pBH6843 KO DHODH SEQ7
ccgagcccacattctccaatggagtggaggcagaggcgggcccagtggcagaaggagcatggcgtggagacagatgagagtgagtctgttgcgggtgcttacgcttgttcggaaaacaggttgggagtggacgaggctgggagattgaaaggctggggcccttgcagtgtgggctgcatgtgtgctcagctaggggcatgcaaaaagcaagcgtgctgggcagaggctgagttgattgtgagagatcgcgggcttttttttttttttttttcttaaactgagctagtatcgggcccctgtgagcacatggtggctagcattatggaaaggatccagggcggaatgaaataagacacgcagccacccttccagataaagtgtggttagaatgggagtcccgtgcgaagagtccgtagattgtgtccctggcttgggaaagagtgcgcagatattgtttcttgacacgtgagaatttctccctccagaggagggagaatgaatacttggtttgctgtacaggcaaatctgatcacatcctctacttccttatttagtggacaaatcccattaaaaatataatcactgattgtggtgaggggttgtgctgtgacatgggagctggaaccgaactctgcacttaaccactgaaccatctccagcccccaaatctgtattttggctgacacccccacatttctcctaccttactttaagaaatgctttccttttagttccaaacagacctgtcttcctctaccccattctctggcccttctcattggcttcagccacctagagattccttctccagctgcttcctcctctttagcttttgtgtctccttggaaagtcaaccttagcctggaaggagcctcaagatccttccattacttatctcttcgtgtcagttttcttgggtttgtgtttacatggccattaatttctctcttcattagatagattacacacttctgaaggacagggacctggtgtggtttgcttgcctttggtgaaggattgaatgaatgcattagccacttggcatctggcagtgataattatcaaaaagcattgtgagcctcctttgaactagggtagtgattctctacccagagtgtgaagctatgtttgtattacaaccacttttatattatacacataggacatttcaggccagtaacttttctaggtataattttaaaatatagacaccatgtcctaactacagtataaaggagaaatgaaaacatgtatttcagtatgtagaagtcagaacacagttcacctacatagatggccaggtgtttaagcctctatttagaaggtgtgcgttggtatacaaacagcactgtataccctttctggtggggttttaggaacagtgaccaagtcttagtaatgttttgtgcaaactgtacaattgtccttaaattacaaggtatctttatttctgtaaaagtcaccctgtacatgtaaaccatgtggttgtgtggtgaactatagcttgcttcttgcctctcctattatcctcagataataggaagttttcctcacataaatagcaatagcaagttcaaacatcatacagtacatagggaaactagtgtgttagctttaattaaagaagaatattgacaggactgatttctccacaccaaatgtattagcatcattccctcattaactagtaaaaattttcccatgtgacccctagggggcagtactgcctgtcttgaaaattccctgcctggtccttaggaaaatattcagggctagaacccatgtaagcagtgtaggtactgcatctacctttgtagatgtgtaagtgggcaggatatgaagggggacagtgtgagcagggaaggactgtcactttgtgtagttgttatgtcctctgggcaggtgtgaagggtcaggaagggtactgcaggctggtctgatggggttccccatggggccttttctctcccccactagaagcgggccctggatgcagccatcatccttgggggaggaggacttctcttcacctcttacctgacagccacgggcgatgaccatttctatgctgaatatctgatgccggccctgcagaggctgctagacccagaatcagcccaccggctagctattcgcttcacgtccctggggctccttcctcgagctacatttcaggactctgacatgctggtaggtcccccggtcaccctgtgttacatttgtgtttgtaggggaggtcacatccttcagcacttcggtattcctctgctgccactgggcttttgaaaaccagagctgcaggttcacaagcagctgggacctggagcccagcccgaggaagggacttttcttctgtgttacaccctgtacttacagaacagcactcagcatatagccggtgcttacagctttaatcctcacagataccctttgagggaggtcctatctcatctccatctacaaatcaggaaactgaggtacagactaagtaagtgacttgcccaaggtcacacagctgggaggtggcaggaccaggattcaaacctatagagtttgactccagtgtccaaccttggtcactggcctgccttgctgagatccctctgctgaacaggaacatcttctggagtcattaagcagctactggatgcaggggacagggtcagcagggaagggctgtcacttgtagatactgtgtcctctgtctggataggtgtgaagtctcagagtgggtgctgcagcctggcctgatgggtccgtcctttccccccatcagaagcagaccctggctgtagtcatcaccctgaggggtggaggacttaagtcctaggcaacctcctgccccagccacattcagccacaactcactcctgtggcccacctggcaccatttataacagagccagtgtggcccttctactgtctctctgaatgctccccttttgagatgggcctaggttgtccaggttggtctcaaacttggggtcccaaatgatttcagaatctcagcttcctgagtaagtgggatcacacagtatgcaccactgtgcgcagtggtccctgttccccgatagccaggccggttgatactcttagcccgattcacctttctcggttttctaagtcttcagttttctatcatgacgagactctcctgggggagggggatggctgggtgcttctggaatgcttggctgacccggtctcctgattgaccggttttaccataatctcaaagaagcctgacatcaacaccccaggctctgtcacacagccagggatgagaactggcttgagggtagcctcaaggaaggcctgttctagctgaacttctcgcctcatggttatgaagtgctgcgtgcacatttttaccttccttgtgctcattctcgtctcctgtggattttgagagcatgtagctttccccttggggactggcctctaagagctcactggcagcaccattgcctgccagtgtccacccttcagctctccatggtgcccatgggctggcttcttgacagttatggaggaagggccagctagggcttgtatgctaggctggctacaggctacctcaaggctggtgacaccaaggactccttctcctgcccaggttgagtagataggaagatacacagtaattgtgcaagacagcacctgtctcctcttcacttgtggtgggacactatctttctctccccactgccttgagaccccctggtgacagactccagcagacatcagaagcacctgcagaatgctgatgcagatagataccccagggtgtccttcctcccaaagatccctattttctgggcccagtgatgcttagcaagctccaggggaattcttatacagtatgctgggatccctgctgtgagaaccacttggtatagctgcttatacctctgacctgtctccttcccaggaagtgagagtcctgggccataaattccgaaatccggtagggattgctgcgggatttgacaagcacggggaagctgtagatggcctctacaaactgggctttgggtttgtcgaggtaggaagtgtgactccccagcctcaggaaggaaaccccagacccagagtgttccgcctcccggaggaccaagctgtcattaacaggtaggtggtggctcaatgtcatagggacatctcctcccctgctgggatctctgagatggaacctgttttgtgcttttctcatatgatcagtggacagtctgtcctttgggatagtcaggagcacctttgaacacctgttgtgtactaggcagctctcgccccaaccttgggaaacagctgttaggattttaccaggtattcccactgaggctctgagagctggtgctggttgcaaagaacagcttgggaaggcttgggctgttgggcttcagtgtgagcttttttacattgttgctctattgcctttgtccaatgttggctaacaggaatataatgatctcacatgtaatttgaaatattctaatgatgcattaaaaactagtgaacttgataatacatttataattattatatttttaattattatgatttaattataaacagtgtgttctaaagtcattttaacctgcagtcaatgtaaaaatcattggttaactatcgtcctctttttattggtttccggtcccccaatgcctttacttctggttcctctcacttggccagggctggtggccacaagcttcagcagcgttggtactgtacaggtgacccttgctttcaatgaacagggacatggtattcaaatgtacagctgctcttaggaggagaatccttcgactgtatgaagccttgcggtttgttgttctgtatagttagtataactgcaaagggaagaccttcgtactttttgctaggagatttttggagaacctccttgtggggattttggcaggcctgtggcagtgcttcctactgcttgtttcaggaaactgatttacaagtcatagatctttctgttacattacaggcagggactgatgtctttaggactggccagacaaaatacttgtgtttctgatttggctgttacaagtgacttcgggtcttaggatgatggtacttgggacagggagtggtgagggacaggcacctgtgctcttgggcatgtgcgaacttagccttcttgctcatatacacagtgtgtgttcagtataggcatgctaacggatgggtatttacacctgcagacccacatgccacaatccatgcagtgttgctctggctgcaagcaacaaagtgatgtaaccagatctcatttgttatcattcttgtcactagcacaaaataactgacagcaggcagcttaaggaatggggtcaggtattttggctcacagtttgaggggacacgccctcccggtggcaggagcctgaggcagagggtcactctgtacctacagtgaggaagcagcaagggaaggatgctggtgcttgggtctctttctccgtcttgctcagctggggtgtgaatccatggtgctgcccatgtttgcggtgggtcttccctgctccattcaaccttcccagaaacagtcttccagacacacaacaggtgtgtttccatggtgactctaagtcacatctagttgacaatgaagcataaccagtggtgagagcatggaaatggtctcaggtacgttttccaaactgccaccttttaattccaccccttacctgtgggtttatgtgctccaggtacggattcaacagccacgggctctcagtggtggaacacaggctacgggccagacagcagaagcagaacaagctcactgcaggtaaactcaggtgttgtgggagggacttactaactctattacaaagaaacatggggagggcatgggattcagcaataagaaacaaatgagcaaacaattaaaaccccacagaacaactcaggggattgtccagcttctaccacagcctcaaaggtctcaaccagatggcataattcagcaaaaccttgctggtctctggcatccatggaacctgaattgtgtcttaacttaggggcttgaagatcagcagagagcatgtgtggagctaagatgcgccccgagttcatcttcccacatcccgccctgctgctgtccttctgttcactgtgtaaatagtgtgtattagttctggaagagctacagaagagaatagagttgtcacactcctgtccttccactcaggggaccagctgtcctcaaatctcacttcggaaacaacctttgcttttggtggattctcatggagacgctccagtttgtcctctgtggtctgcatggctctctgaagtgcattttggggtcaaagccctgggtggtggcccccctccccatgtctccctgtgtggcttctgcagtccatggagatttttctcctttgcctctggaatgtctttcaggaggtcttagtctcatttgatgtccccatagtgtgacaattaagccaaggacttctgcatttatttgaggagctaaggaagagagggctgaagcatttgacgagtttagagggtgggaacaggaaatgacaatgtttaaaaaaacccctggttttgacggaaccgggtctgccagccctgtagaaccttgaacacaatgtttgtggtttgtggcgttctcctgcctcctgccttccgtttcttcgttttaatgccttctgtgggctaggtttattgccattgtcctgtgtccacccttcatcctcattctgtgccctcacagtcactggagtgaggccaagttctgtgtctttgccctgcctacatgtgtctgctgacagctagcagcctcatagaaacttttcatcagcaccatgcctaggaaccctagtggatagaagagactgtgctttgtgtaaagtgtagttcagccttcctgactccagaactgtgactgtgggcaggtgaccactaatgaaaggctcagttgcctcttggaagccatactctcaatccagtttacttgtgctaaagcttacagtgatcctggcttgctgggtgctagacttgaagctttgagaccttgttctgtatatagtctaatccctggctccacccagcccacttaggaaattagttacacaaatcttacttttaagttgatgacccagaagatgacgggttgtgagagatggactgtgagaagggggctagcaatacagtgggggatgttgcccgtgtcctccctggcctggtatgggtgagctgacttggtgttctaggtctggctggattggcagatggacagcagcctgggccactgacatactaggagttgtaagaaagttgagttgtaataaagatgaatccaggaaactcctttctgccaaagagaacatgagtctgaaagagcatttttctagaggcttggccttttgagagtgacagggggcaggtgtgagtaattacacccaggccccaggagtgtcttgaggctacagagatgtatcatcaccctaattataagttcttttctcagagaacaagaaagatttattacacacttccatctactttttaggcatgatagttgaaaacatttcctagtgttttcctgtgtagctcaggctggcctcagacttacagcaatcctcctgcagactaaatttccatgtgtggcctccagtgttttatacttttgtttttaatcatttcacatacagtcccttgaccaaggctcatgagattcaggttgttcttgctgacatgcccatcaatacctgcctactctctcttttgttatctctcaaaccactgatctgtgaatatagcaagtgtcattgggagtcattttattgctacatacttcaagaagagcagtagtatttgtttttttccccatgtccctgatttgtctggactcagatccttggccacccatgcagtcagtgttggggatgggttccatctcatggattgggccttaaatacaatcagattctggttggttactcccgcagctttgtgctactgtttcactagtgcatccagggcaggtcatcattgtagatcaaaagatgtgtagcggggttggtgtttacctttctcctttggtaacatgcagaatacctcccagtaccatggacaccaccagagggatgaaggctgtaggtaggcaccagctcgacttctccctatttaataacttgtgtaggtgttgtctttagcaatagagccttgtcagttttcagagagcaaccaatatccttgacaatagcctgggttgtttgggtattctcatggggcccctttggccaacaacttctttgaaagtctggtcaaattcttcactaaaaccatctggcactgggcattttttggttgggaggcttttatgactgcttctattttactaggggttataagtttgtttacattgcttatccgatcttgatttaactttagtagatggtatgtatcaagaaaattattcatttattttcaattttccatttaggtagagtataggtttttaaaacacatccctatgattctttggatttccttggtgtctgttgttatgtcactcttttcatctctaattttgttaatttggatctttcctctttgccttttaattaatttggctaagggtttgtcaatcttactggttttctcaaagaaccaactcttcgtttcattgattctttgcattatttttgtctgtttctatttcattgatttcagccctgagtttgattatttcctgccatctactcctcctgggtgtgacttcttgttgttctagagctttcaggtgtgctagtatgaaatctctctaatttatgtaggcacttagtgctacataaagttttgggtttttgttttgttttgacctatttttcattcagtagtgagttgttcagtttcagttgttcagtttccatgagtttgtaagctttctgttgtttttgtaggtgttgatattcagctttaatctgtggtggtatgatagggtattatttcagttttcttgtatcttttgagacttgctttatggcctagtatatggtcagttttggagaaagttccatgaggtgctgagaagaaacgttttgtgtttgggtgaaatgttctataaattaggtccatttggtttaacacatcatttagctccatcatttctttgttcagtttttgtctggatgacctgtctattgtcgagagttggggagtatcaaagtatcccactatgtgtgtgtgtgtgcggaggggtcaatatgtgatttaagctatagtagagtttcttttatgaacttggatgcctttgtgcttggtgcatagatgtttagaatttcaatatcctcttggtgggtttttcctttgatgagtatgtagtttccttccctatctatctcttgattagatttgatttgaaatctattctgtcatatattaaaatggcttcacccatttgctttcttgtccatttgcttggaatatctttttccatccttttactctgaggtgatatctatccttgatgttaaagtatgtttcttggattcagttaaagaatgaatcctatttttgaacccaattttttagtctgtgtcttatttattgggaaattgaggccactgatatcagtgtttgttgattcctgttatattattgttatggcgtaggccccttcccttttgatttgctggtctgagattatttattcaggctgaagttttccttgtagtaccttctatcaagctggatttgtagacagaaaccacttaagtttcattttattgtagattgtcattctttcttcatctctgtgattaaatgttttgctggctatagtagtctgggctggcatctgtggtagaatgtctgcccaggacctttgacttttagagtctcgattgaagtcaggggttattctaataggtttgtctgccgttatatgttatctggtctttctctattgtggcttttggtattctttctttgttctgtacattctgttttttgattattatgtgttgtggggaatttatttttggcccagtccgtttggtgttctatttgtttcttataccatgataggcacttccttctttaggttaggtaacttttcatctgtgattttgttgaaaatattttctgtgcctttgacctgggtttcttctccttttgctatccctgttacttatagatttttggtgttttcatagtatcctagatttcctggatgttttgtgcctggattttgttttctttctttttttgtagatttaacattttctttgactgcagtatccttgtctcctatcttgtcctcagtgcttgagactctgtcttccatttcttgtatgattttggtgaggcttgcttctaagatttctgttctagttcctaaatttttcatttccagctttacctcaatttgggttttctttagcaattccatttcctctttcatgtgttgaacaattttcttcatttcattgcactgtttgtgttttcattaatgggtttattcatatcttctttagggaccttgaacatattcataatagctattctgagagccttgtcttatgcttccctgtattgcatttctcggagcctgctgtggtagggttgctgggctctagtggagacatgtcgttctggctgttactgggtttttacactggtgtctaggcgactgggtttgagaagattgtaattctaggtgctgatatctggtcttgtttttgttggggtgatgttcagttccttggtttctgttgcccccccccctcagggggggtgtggtaactggattggttgcctggtagggaatgcttctgagatcctgccagaaccctgccactggcagtcttgggtagaaagtgtttctaggtgttgggagctgacactaatgattgaggatgggttagaagcagtggtggcgggagagtccacaggaggaggagagctgggtgtgccaccagggtctgcacagaggcctgggaatgagaacagagatgaaggtgaggcctcagcaggtagtctgctacaaggttgggataaggctgggagattggaacttggggacaggagggagagtgaagatcgcagacccatcccctggccaggtgggggaagcctggaggagaagatctgtgtgatctgctggaaatgggtcccttagtaacttcttgaagtttctttgattttgaggctgctgttgggggtcccctgtatgccaagcatgtggtatatcactgagatagaatctccatagccctgcttcttttttgagactgggtctcatatcggccaggttggccttgaactagctatgttgaccttgaacttttccttacctatacctgagaactgggattacaagtgcccatcacacccagcttcctattgtttttgcttttttcctagtatttaagcttctggcttccccattaaaatttaaaagatgaaaggcttagtacacgggaagcatccttgaaggtgcacacacttgccatatagagaggatgaagtggttctaagtcatcaggcagcagccccaggatcagacagttcacattctccatcatctggttcaggggagccccacctgtactctgaatgttgcctgggaaactgtggggacacactcttgatatttacagatgggctgcctctgggaataaacctggggaagaataagacttcggaggatgctgctgcagactatgtagagggtgttcgtgtcctgggccccttggctgactacctggtggtgaatgtgtccagtcccaacactgctggtctgaggagcctacagggaaaggctgagctgcgccgcctgctggccaaggtgtgtcattacaccatcacatgcctgttgtccttactccttttcattcttcaggtgaagattcaggacaactgaggagaaactgttcttcacagctggcctaggagccctcatcacacattttccaagtaccctctcatgtctcacagccccggtcatacacaatagacagttcactgctttaaaaccacaggcaagcagagcagagcaggcggggctcccatgtatcactctgtccccagaactgtgaatgctcagcacttgtgacacacctccttgtttgttttcaggaacaaaatcaaaacccttgagcagttatctcggcggggggtgcgggggtgggggaattgctggtgctttagttgaccttaggtgaaaatgctggcctgcactgcggggctatgggctgggtccccatctctggcttgtcaacctaggtgctgcaggagagggacgctttgaagggagcgcagaagccagcagtgctggtgaagatcgcccccgacctcacggcccaggacaaggaggacattgccagtgtggcgagagaggtttgagttggggtggtccagggcagggtgggggtagccttcatcgtccactgctgctgggataacacagaagggcatgattggtgacttcctctgtgtgaagtggacagctggttgattgtctgtcattgtatagttcatctggtagcaaacagtgagtttgaaaatgtgtttggtgagtctttttcttgcttctgatctgtcttcatccagaaagtctgaggcctgtgctagtctctgccagtctcacctgggacttagaatggtgtctgtccctttccagcttgtgtaaacaccaggcttctctggctaaaaaggtagtaggaacacagtctgctgttctggacttcagtcttgttctactgtgtactccctgagatactcacagacagcttgttctaagggtcaaactctgtgtaggcactgtgatgggttcagcaggagatgctgctgtgtcttcagcattgagaggctaattctgatggcttctccaatcaagatgtaggtgaggcctgtgagggtcttgctctgcagagctggcccctggcctggtggctgcttcaatcctcaaaagacagtttccttgagtacttcagatccatggcttaaggctctttttctgtcttgtgctgcagctgggcattgatggattaattgtcacaaacaccacagtgagtcgcccgactggcctccaaggtgctctgcgttctgagatgggaggactgagcgggaagccactccgagatctgtcgacccagaccatccgggagatgtacaccctcactcaaggtaaggcttttttgtttgtttgtttgaggcaggatttctctgtttaacacctctggctgtcctggaactcacttggtagaccaggctggcctggaactcacagcttccctagtgctgggattaaaggcatgtgccaccattgcctggctaaggcaagacttctttggacaaatgtgaggtcctggatcttccctcattcactgtgtttgctgagaactctggttctgccctcatcggctgtgtttgctgggactgaggcctgatggagccctgggtctttagccctcccttcccggccttgctatgtgcttctctccaggcaggattcccattatcggggttggtggtgtgagcagtgggcaagatgcgctggagaagatccaggcaggggcctccctggtgcagctgtacacggccctcaccttcctggggccacccgtcgtggtcagggtcaagcgtgagctggaggcacttctaaagtgagtagggttcgatgcagctgagacgtagaaagtgacacttgtcatcagtctattgtgtactcccagagggccggagggaacactgagggcatggtgggacgatttctctgctgcagctttggccaaggacaaacagtgccagaggaattcagaatgcttctgaggcagggctcattacaaggcaggacttgccacttgcccaggggctgggcatggaggatgaagtagtaatttacattgactcagtgtctggaagctgcaggttataaagtcacttcccttcctgcacagaaggcctggctgtacatatgtgcaggggcctgggtgagggcagagtagcagtggttgtaaggtgtgttgggtgggacggtgtggtaagcggtgtgctcatggtgagtgtgggcttccttaggacaggctatttgttttctgtccagagagcggggttttaacacagtcacagaagccattggagcagatcatcggaggtgacggttcctgccagatgccccatccagaacgtgcccaccaactcaagcaagccttgtggctgcatcataagaggaagatctgtctcaagctatgtcccttgactgtgtgacctggctggactgcataagccagtcacggttatcactagacagtaaaggctttctctaatgagaccatgaactctacagtcactttctggatctaagtcctgggatccctcagtattataaggacattggctctttgggaggaaaaatcatggagaaaataaagccatttcaatctgttttcaa

SEQ ID NO: 28 - protein, 395 aa, Artificial Sequence
  amino acid sequence of human DHODH G202A
MAWRHLKKRAQDAVIILGGGGLLFASYLMATGDERFYAEHLMPTLQGLLDPESAHRLAVRFTSLGLLPRARFQDSDMLEVRVLGHKFRNPVGIAAGFDKHGEAVDGLYKMGFGFVEIGSVTPKPQEGNPRPRVFRLPEDQAVINRYGFNSHGLSVVEHRLRARQQKQAKLTEDGLPLGVNLGKNKTSVDAAEDYAEGVRVLAPLADYLVVNVSSPNTAGLRSLQGKAELRRLLTKVLQERDGLRRVHRPAVLVKIAPDLTSQDKEDIASVVKELGIDGLIVTNTTVSRPAGLQGALRSETGGLSGKPLRDLSTQTIREMYALTQGRVPIIGVGGVSSGQDALEKIRAGASLVQLYTALTFWGPPVVGKVKRELEALLKEQGFGGVTDAIGADHRR

SEQ ID NO: 29 - DNA, 18 bp, Artificial Sequence
  corresponding piece of DNA for generating GS gRNA
gagtatgtgaagactttg

SEQ ID NO: 30 - DNA, 20 bp, Artificial Sequence
  corresponding piece of DNA for generating GS gRNA
ccatctttattctcatgggg

SEQ ID NO: 31 - DNA, 5562 bp, Cricetulus griseus
  misc_feature (4467)..(4484): target of GS-1 gRNA
  misc_feature (4611)..(4630): target of GS-2 gRNA
accttccaccatggccacctcagcaagttcccacttgaacaaaaacatcaagcaaatgtacttgtgcctgccccagggtgagaaagtccaagccatgtatatctgggttgatggtactggagaaggactgcgctgcaaaacccgcaccctggactgtgagcccaagtgtgtagaaggtgagcatgggcaggagcaggacatgtgcctggaagtgggcaagcagcctgagatttgaccttccttctgttttgtttgcaaagtctttcaaaagcaggtctcttcaggcctcagtcagtcacccgtaagctgccgagtagtctggaggcatagaaaacaatggaggcctttatttagatggaatcttgtgtgtgctggtacactgaagaaaaatattgggtcatatttgtagggggtgggaggttggagtattgctaacctagccaaccccaggaacctagtttgaaagacctgtaactagaatatgctatcaagtttatagagcagtggttctcaacctttcaaatgctttacacttgaatacaactcctcatgttctggtgattacccccatcccaaccattgctaacttcttaactgaaatttcactactgctacgaatcataatgtatctgtgtttttggatggtcttaggtgacccctgtgaaagggttgtgagaccatcctcaaaggggttgtgacctacaggttgagacccttttgagtgctgtgtttattagtatttatacagtggaattctgggtgcaaagcacatgctccaaagtagtttctctgggactggccatttgttttcagatggggatacttttaaaaacttgcaaaggaaccaaaaaaaaaaaaaatgcagaaaaaaggaggggggggagggcacgcctttaatcccagtacttgggaggcagaggcaggcggatctctgtgagttgaagcccagcctggtctacaagagctagttccaggacagcctccaaagccacagagaaaccctgtctcaaaacaaacaaacacacaaaaaaattaaaaaaaaaaaaaaactttcaaaggagacctgttttattttagttgtggcctttgttttggtaggaagggcagctagtttaggatgagtttttattattctaagatgttgccgtttgagtgaatgaatgaccagatgacagcatataacatgtacttgttacttggcagaagtaggtaggtcgttctgtttctgccttcagctcataggtaactggggagacaaactggccccaaaacaaggaaaaggaacaagtggtaggagagcaactgtttcctcatctacaagagcacagcctgagctacaacagtcaggcccggagagggatgagagaagggaggggatgaggtggcctagtgagggagtcagttttgctctgtgccatgagtgtctcactcactggaagtggtgtcagaatgactggtgcacagtagacttacagagaggactcatctgtttgttgcttgggtggttcttgtgatgcagtgctcttgggaacctcagaaggaggaacatagggataggtgggcatagacatcaggttgtccctaattaatgatgatacatttacatacatgccactcagaagacacagtagattttcagtgatggaaatatgatgagaggctagctgtcttgtgtgtatatttttaataaatttttaataaatttcatgtgtgtgagtcagtgcgtgtgtgcgtttgctcgcccagtgctgtgccagcagaggtctgaggagggtgtgagaatcccaggaactgaagttaacagttgtggttaagagtacttatcactcgttaccagcacctacatggtggctcacaaccatctgtaactccaatttcaggggctccaaccccctcttctgcaggcatacacttgcacagatatacatgcaagtaaaacacccctacacacataaaaataaatacgtcttcttaaaagttaattttccatctttatttggcccagagttacctgagtggaattttgatggctctagtacctttcagtctgagggctccaacagtgacatgtatctcagccctgttgccatgtttcgggaccccttccgcagagatcccaacaagctggtgttctgtgaagttttcaagtacaaccggaagcctgcaggtgtgtatggggtgggcgtgaatgtcttaagaatctagggatggatgatcagatgtccatccttctaccctgaacttgcctgctgaaaaacagtgtggtccgcccctccatggtcccttttattggttgtataaacagtgttgaatcttccatctgtttgctgataggggtccccagtgacagtcttgatctgcttctacatttaaaaagctgtaattcgtacttaagcgttttggggtttaactactagatctgccatttattgccagtgaccttggcatactttgccccatgcttctattttgctgaattatgtgtagagagagacgagacagagcatgcttgaactgagggcgtactgtgctctgtgtggaagtcaaccgacaacctgtggaatcagttctctcctgctgtatttgtagattctggaggtggaactcaggttgccatgagcattatgattcctggctaagctgtttgcccatgaagccttctgtacctgctcatagaattttgtttatgccgtgctatccatactcagttttcagatagcttcttaaacccagggaactctaatttacataaactctcttccagtactgccagtaaggcttggtggccctataccttcagtacctctgttttgaaaaggaagtattgttggtcaagggtatgtacctcagcatggcagccatggggttcctggctgtgccgcttgccctataacctgggcacgtcaccaaacaccctctctcagggcttcattttctcatttgtgaaagtgaagattgctaacactcatctcaaactcagttaaatgataaattgcttttctagcttgggaattgttttcagttacactcacctctccctcgctttctctctcttttttgtaccagccaatactgtgtaatttagcactcagactcacctggaatgtaaacctaatggacaaattattctcagtaaaatgacagctctggccttaagtgcctacgaaactagggaatacgtttgacaagcaggagcagctgtcttgtgaatagagggtggaagtgtctggcatgtggtacttggaaagtggccagcgtgcagataggatgaacacttgttttgctctcactccattcccatgagatttcatagctgactttaattataaaaagtctctcagccttttcctgcaaatgtactatcattgcttcttcacagtggttgggcctgagtaggtccagcctatgatgacttcagctgtgtaagagttgaggacactactccttacagcatgttgatgctttattcctagagaccaatttaaggcactcgtgtaaacggataatggacatggtgagcaaccagcacccctggtttggaatggaacaggagtatactctgatgggaacagatgggcacccttttggttggccttccaatggctttcctgggccccaaggtaagttccccaggtgaaataaaagcttcctccccataagttcttactgtccagagacaggagcagctcccaaatcagcaaacagactggcagctgaaaataacagactgtccttgcatccctcaaatccagatgtgctttgaatttaaagtgacaggatggtgatgagatggctcagtgggtaaaggtgcttgccaccaggcttgacagcccgagtttatccctgagacccatataagttattctctgaccatctgcacatgcatgcatatacaaaaagtgaaaagctattcagagtgggcagtagttctaccaaggctacagcaaagaggaaagacctagcctcctacctgcaggtgaagacaggatgtgcgaaagcaagtcttaggaccttgtcattttctggctttggggggttatggactctgattcttcactgattgctcttgattctccttcaggtccgtattactgtggtgtgggcgcagacaaagcctatggcagggatatcgtggaggctcactaccgcgcctgcttgtatgctggggtcaagattacaggaacaaatgctgaggtcatgcctgcccaggtaaatggcactattctgttccttttcctcccctctgaagacttggcacatggggactttggttaacaagggtgatgacttaaaagtggttcagggtagaggtaagtagaacaagctaggagcttgagttggcctgaacagttagttggccttattctaaaggtcaacatgttctttctagtgggaattccaaataggaccctgtgaaggaatccgcatgggagatcatctctgggtggcccgtttcatcttgcatcgagtatgtgaagactttggggtaatagcaacctttgaccccaagcccattcctgggaactggaatggtgcaggctgccataccaactttagcaccaaggccatgcgggaggagaatggtctgaagtaagtagcttcctctggagccatctttattctcatggggtggaagggctttgtgttagggttgggaaagttggacttctcacaaactacatgccatgctcttcgtgtttgtcataagcctatcgttttgtacccgttggagaagtgacagtactctaggaatagaattacagctgtgatatgggaaagttgtcacgtaggttcaagcatttaaaggtctttagtaagaactaaatacacatacaagcaagtgggtgacttaattcttactgatgggaagaggccagtgatgggggtcttcccatccaaaagataattggtattacatgttgaggactggtctgaagcacttgagacataggtcacaaggcagacacagcctgcatcaagtatttattggtttcttatggaactcatgcctgctcctgcccttgaaggacaggtttctagtgacaaggtcagaccctcacctttactgcttccaccaggcacatcgaggaggccatcgagaaactaagcaagcggcaccggtaccacattcgagcctacgatcccaaggggggcctggacaatgcccgtcgtctgactgggttccacgaaacgtccaacatcaacgacttttctgctggtgtcgccaatcgcagtgccagcatccgcattccccggactgtcggccaggagaagaaaggttactttgaagaccgccgcccctctgccaattgtgacccctttgcagtgacagaagccatcgtccgcacatgccttctcaatgagactggcgacgagcccttccaatacaaaaactaattagactttgagtgatcttgagcctttcctagttcatcccaccccgccccagctgtctcattgtaactcaaaggatggaatatcaaggtctttttattcctcgtgcccagttaatcttgcttttattggtcagaatagaggagtcaagttcttaatccctataca

SEQ ID NO: 32 - DNA, 56 bp, Artificial Sequence
  GS1_F primer
acactctttccctacacgacgctcttccgatcttggccttattctaaaggtcaaca

SEQ ID NO: 33 - DNA, 52 bp, Artificial Sequence
  GS1_R primer
gtgactggagttcagacgtgtgctcttccgatctcattctcctcccgcatgg

SEQ ID NO: 34 - DNA, 1417 bp, Cricetulus griseus
ccgagccgagaatgggagtagagccgactgcttgattcccacaccaatctcctcgccgctctcacttcgcctcgttctcgtggctcgtggccctgtccaccccgtccatcatcccgccggccaccgctcagagcaccttccaccatggccacctcagcaagttcccacttgaacaaaaacatcaagcaaatgtacttgtgcctgccccagggtgagaaagtccaagccatgtatatctgggttgatggtactggagaaggactgcgctgcaaaacccgcaccctggactgtgagcccaagtgtgtagaagagttacctgagtggaattttgatggctctagtacctttcagtctgagggctccaacagtgacatgtatctcagccctgttgccatgtttcgggaccccttccgcagagatcccaacaagctggtgttctgtgaagttttcaagtacaaccggaagcctgcagagaccaatttaaggcactcgtgtaaacggataatggacatggtgagcaaccagcacccctggtttggaatggaacaggagtatactctgatgggaacagatgggcacccttttggttggccttccaatggctttcctgggccccaaggtccgtattactgtggtgtgggcgcagacaaagcctatggcagggatatcgmggaggctcactaccgcgcctgcttgtatgctggggtcaagattacaggaacaaatgctgaggtcatgcctgcccagtgggaattccaaataggaccctgtgaaggaatccgcaggagatcatctctgggtggcccgtttcatcttgcatcgagtatgtgaagactttggggtaatagcaacctttgaccccaagcccattcctgggaactggaatggtgcaggctgccataccaactttagcaccaaggccatgcgggaggagaatggtctgaagcacatcgaggaggccatcgagaaactaagcaagcggcaccggtaccacattcgagcctacgatcccaaggggggcctggacaatgcccgtggtctgactgggttccacgaaacgtccaacatcaacgacttttctgctggtgtcgccaatcgcagtgccagcatccgcattccccggactgtcggccaggagaagaaaggttactttgaagaccgccgcccctctgccaattgtgacccctttgcagtgacagaagccatcgtccgcacatgccttctcaatgagactggcgacgagcccttccaatacaaaaactaattagactttgagtgatcttgagcctttcctagttcatcccaccccgccccagctgtctcattgtaactcaaaggatggaatatcaaggtctttttattcctcgtgcccagttaatcttgcttttattggtcagaatagaggagtcaagttctt

SEQ ID NO: 35 - DNA, 16 bp, Artificial Sequence
  GS F primer
acctttgaccccaagc

SEQ ID NO: 36 - DNA, 17 bp, Artificial Sequence
  GS R primer
cgtcgccagtctcattg